European Patent Application EP 4 678 769 A1, published January 14, 2026. Title: USE OF PLASMA CELL-FREE DNA METHYLATION MARKER IN LIVER TUMOR DETECTION. Applicant: SINGLERA HEALTH TECHNOLOGIES (SHANGHAI) LTD. The sequence listing filed with the application follows.

SEQUENCE LISTING (81 sequences)

SEQ ID NO: 1 - DNA, 24 bp, synthetic construct
  source 1..24: mol_type = other DNA
gacgacgtatttttttcgtgtttc

SEQ ID NO: 2 - DNA, 16 bp, synthetic construct
  source 1..16: mol_type = other DNA
gcgcacctctcgaccg

SEQ ID NO: 3 - DNA, 27 bp, synthetic construct
  source 1..27: mol_type = other DNA
tttgtatcggagtagcgattcgggagg

SEQ ID NO: 4 - DNA, 20 bp, synthetic construct
  source 1..20: mol_type = other DNA
gtagttggatgggattattt

SEQ ID NO: 5 - DNA, 17 bp, synthetic construct
  source 1..17: mol_type = other DNA
cacccgcaaaatcctct

SEQ ID NO: 6 - DNA, 18 bp, synthetic construct
  source 1..18: mol_type = other DNA
ttgttgcggtcgcggacg

SEQ ID NO: 7 - DNA, 23 bp, synthetic construct
  source 1..23: mol_type = other DNA
aaaaaaaaaaaaactccacattt

SEQ ID NO: 8 - DNA, 17 bp, synthetic construct
  source 1..17: mol_type = other DNA
tagttgnggagtttggg

SEQ ID NO: 9 - DNA, 23 bp, synthetic construct
  source 1..23: mol_type = other DNA
atcgtacgtaaggttcggagcga

SEQ ID NO: 10 - DNA, 17 bp, synthetic construct
  source 1..17: mol_type = other DNA
cgtcgtacgtcgttcgt

SEQ ID NO: 11 - DNA, 17 bp, synthetic construct
  source 1..17: mol_type = other DNA
gatcgacgcgactcgac

SEQ ID NO: 12 - DNA, 21 bp, synthetic construct
  source 1..21: mol_type = other DNA
cgttgttgtttggcgacgtcg

SEQ ID NO: 13 - DNA, 17 bp, synthetic construct
  source 1..17: mol_type = other DNA
gcgcgggaggattttcg

SEQ ID NO: 14 - DNA, 18 bp, synthetic construct
  source 1..18: mol_type = other DNA
gcatcacgtcctctcgcg

SEQ ID NO: 15 - DNA, 20 bp, synthetic construct
  source 1..20: mol_type = other DNA
cgatttcggtcgtttatggt

SEQ ID NO: 16 - DNA, 22 bp, synthetic construct
  source 1..22: mol_type = other DNA
gcgttttagttagatagggcgg

SEQ ID NO: 17 - DNA, 18 bp, synthetic construct
  source 1..18: mol_type = other DNA
gaaccccttccccgaaac

SEQ ID NO: 18 - DNA, 19 bp, synthetic construct
  source 1..19: mol_type = other DNA
gcggcgcgtagttttaggc

SEQ ID NO: 19 - DNA, 20 bp, synthetic construct
  source 1..20: mol_type = other DNA
tttcgaagttttcgggtgcg

SEQ ID NO: 20 - DNA, 19 bp, synthetic construct
  source 1..19: mol_type = other DNA
cgaaaaccgccgacactta

SEQ ID NO: 21 - DNA, 19 bp, synthetic construct
  source 1..19: mol_type = other DNA
tgcgtcgatattcgatacg

SEQ ID NO: 22 - DNA, 18 bp, synthetic construct
  source 1..18: mol_type = other DNA
gtgtacgcggcgtggagg

SEQ ID NO: 23 - DNA, 20 bp, synthetic construct
  source 1..20: mol_type = other DNA
acgcacctttcgacgaaaca

SEQ ID NO: 24 - DNA, 20 bp, synthetic construct
  source 1..20: mol_type = other DNA
tatcgcgcgttcgtcgtgtt

SEQ ID NO: 25 - DNA, 17 bp, synthetic construct
  source 1..17: mol_type = other DNA
ggttgcgagttttaggg

SEQ ID NO: 26 - DNA, 17 bp, synthetic construct
  source 1..17: mol_type = other DNA
cacgctcacacactatc

SEQ ID NO: 27 - DNA, 19 bp, synthetic construct
  source 1..19: mol_type = other DNA
cgtgagcggattcgagggt

SEQ ID NO: 28 - DNA, 16 bp, synthetic construct
  source 1..16: mol_type = other DNA
gggggttcggttagag

SEQ ID NO: 29 - DNA, 23 bp, synthetic construct
  source 1..23: mol_type = other DNA
aaactaaccaaaataaaaatcca

SEQ ID NO: 30 - DNA, 17 bp, synthetic construct
  source 1..17: mol_type = other DNA
ttgttttcgcgcgggtg

SEQ ID NO: 31 - DNA, 17 bp, synthetic construct
  source 1..17: mol_type = other DNA
tagagggcgttagggaa

SEQ ID NO: 32 - DNA, 19 bp, synthetic construct
  source 1..19: mol_type = other DNA
ccccctacccatttaattt

SEQ ID NO: 33 - DNA, 21 bp, synthetic construct
  source 1..21: mol_type = other DNA
tcgttcgagttgtagagacgc

SEQ ID NO: 34 - DNA, 21 bp, synthetic construct
  source 1..21: mol_type = other DNA
cgttcgttacgtcgttttcgt

SEQ ID NO: 35 - DNA, 17 bp, synthetic construct
  source 1..17: mol_type = other DNA
gatcgacgcgactcgac

SEQ ID NO: 36 - DNA, 22 bp, synthetic construct
  source 1..22: mol_type = other DNA
cgttgttgttttggcgacgtcg

SEQ ID NO: 37 - DNA, 21 bp, synthetic construct
  source 1..21: mol_type = other DNA
ttgaggaagttttgcgtacgg

SEQ ID NO: 38 - DNA, 16 bp, synthetic construct
  source 1..16: mol_type = other DNA
cgaatcccgcgcgaat

SEQ ID NO: 39 - DNA, 16 bp, synthetic construct
  source 1..16: mol_type = other DNA
ggggttagcgcggcgg

SEQ ID NO: 40 - DNA, 18 bp, synthetic construct
  source 1..18: mol_type = other DNA
tttttgttgggcggtcgc

SEQ ID NO: 41 - DNA, 19 bp, synthetic construct
  source 1..19: mol_type = other DNA
accgaaccgtcgacgctcg

SEQ ID NO: 42 - DNA, 17 bp, synthetic construct
  source 1..17: mol_type = other DNA
cggtcgagggcgggtcg

SEQ ID NO: 43 - DNA, 15 bp, synthetic construct
  source 1..15: mol_type = other DNA
tagttcggggcggcg

SEQ ID NO: 44 - DNA, 16 bp, synthetic construct
  source 1..16: mol_type = other DNA
ccgccacatcctaccg

SEQ ID NO: 45 - DNA, 15 bp, synthetic construct
  source 1..15: mol_type = other DNA
tgttcgcggcggcgg

SEQ ID NO: 46 - DNA, 22 bp, synthetic construct
  source 1..22: mol_type = other DNA
cggtcgaggtggttttataagt

SEQ ID NO: 47 - DNA, 18 bp, synthetic construct
  source 1..18: mol_type = other DNA
acgcgaaaacaaaacgcg

SEQ ID NO: 48 - DNA, 20 bp, synthetic construct
  source 1..20: mol_type = other DNA
tgtggttcgtttcgggtcgg

SEQ ID NO: 49 - DNA, 22 bp, synthetic construct
  source 1..22: mol_type = other DNA
gcgttttagttagatagggcgg

SEQ ID NO: 50 - DNA, 20 bp, synthetic construct
  source 1..20: mol_type = other DNA
gaaaaccccttccccgaaac

SEQ ID NO: 51 - DNA, 19 bp, synthetic construct
  source 1..19: mol_type = other DNA
gcggcgcgtagttttaggc

SEQ ID NO: 52 - DNA, 23 bp, synthetic construct
  source 1..23: mol_type = other DNA
gatacgttggcgaatttttcgtt

SEQ ID NO: 53 - DNA, 18 bp, synthetic construct
  source 1..18: mol_type = other DNA
cgaaacgaaaaaccgcgc

SEQ ID NO: 54 - DNA, 28 bp, synthetic construct
  source 1..28: mol_type = other DNA
agatagtatgttgtttagtagcgtgcgg

SEQ ID NO: 55 - DNA, 15 bp, synthetic construct
  source 1..15: mol_type = other DNA
cgtgggaggagcgcg

SEQ ID NO: 56 - DNA, 16 bp, synthetic construct
  source 1..16: mol_type = other DNA
aatcgaccgccccaca

SEQ ID NO: 57 - DNA, 19 bp, synthetic construct
  source 1..19: mol_type = other DNA
ggcgagattcggagtcgcg

SEQ ID NO: 58 - DNA, 23 bp, synthetic construct
  source 1..23: mol_type = other DNA
gggaagataaacgacgttttgaa

SEQ ID NO: 59 - DNA, 22 bp, synthetic construct
  source 1..22: mol_type = other DNA
aacccaacaacgctaactaaac

SEQ ID NO: 60 - DNA, 22 bp, synthetic construct
  source 1..22: mol_type = other DNA
tacgtttcggtatttcgcggcg

SEQ ID NO: 61 - DNA, 24 bp, synthetic construct
  source 1..24: mol_type = other DNA
gttttttttcgattttttataggg

SEQ ID NO: 62 - DNA, 25 bp, synthetic construct
  source 1..25: mol_type = other DNA
aaccgaaaaaaaaaataaaaaactc

SEQ ID NO: 63 - DNA, 22 bp, synthetic construct
  source 1..22: mol_type = other DNA
tgtttttttttcggcgttcgcg

SEQ ID NO: 64 - DNA, 20 bp, synthetic construct
  source 1..20: mol_type = other DNA
gttgtacgcggcgttggagg

SEQ ID NO: 65 - DNA, 20 bp, synthetic construct
  source 1..20: mol_type = other DNA
acgcacctttcgacgaaaca

SEQ ID NO: 66 - DNA, 20 bp, synthetic construct
  source 1..20: mol_type = other DNA
tatcgcgcgttcgtcgtgtt

SEQ ID NO: 67 - DNA, 16 bp, synthetic construct
  source 1..16: mol_type = other DNA
gggggttcggttagag

SEQ ID NO: 68 - DNA, 23 bp, synthetic construct
  source 1..23: mol_type = other DNA
aaactaaccaaaataaaaatcca

SEQ ID NO: 69 - DNA, 17 bp, synthetic construct
  source 1..17: mol_type = other DNA
ttgttttcgcgcgggtg

SEQ ID NO: 70 - DNA, 25 bp, synthetic construct
  source 1..25: mol_type = other DNA
gtttgtattttttgtagtttttaag

SEQ ID NO: 71 - DNA, 22 bp, synthetic construct
  source 1..22: mol_type = other DNA
ccnactctactaaataaacatt

SEQ ID NO: 72 - DNA, 22 bp, synthetic construct
  source 1..22: mol_type = other DNA
tgttgtatttcggcgtttcgcg

SEQ ID NO: 73 - DNA, 20 bp, synthetic construct
  source 1..20: mol_type = other DNA
agtttgcgcgttttgcgagg

SEQ ID NO: 74 - DNA, 22 bp, synthetic construct
  source 1..22: mol_type = other DNA
aacaaaccccgaacaaataccc

SEQ ID NO: 75 - DNA, 21 bp, synthetic construct
  source 1..21: mol_type = other DNA
taggcgcgttttcgttttacg

SEQ ID NO: 76 - DNA, 22 bp, synthetic construct
  source 1..22: mol_type = other DNA
agatggtcgagcgttttttacg

SEQ ID NO: 77 - DNA, 21 bp, synthetic construct
  source 1..21: mol_type = other DNA
aactaacgacgacgctcacca

SEQ ID NO: 78 - DNA, 22 bp, synthetic construct
  source 1..22: mol_type = other DNA
tcgcgggttattttcggtttcg

SEQ ID NO: 79 - DNA, 21 bp, synthetic construct
  source 1..21: mol_type = other DNA
tgcgtaggtttggtggtgaag

SEQ ID NO: 80 - DNA, 22 bp, synthetic construct
  source 1..22: mol_type = other DNA
caacgaacccgaaaacaaaccc

SEQ ID NO: 81 - DNA, 21 bp, synthetic construct
  source 1..21: mol_type = other DNA
acgatacgttggagtcggtgc